European Patent Application EP 4 617 287 A1, published September 17, 2025. Title: 补体抑制杂合蛋白突变体及其抗体融合蛋白. Applicant: 天辰生物医药（苏州）有限公司. The sequence listing filed with the application follows.

SEQUENCE LISTING (97 sequences)

SEQ ID NO: 1 - protein, 381 aa, artificial sequence
MTVARPSVPAALPLLGELPRLLLLVLLCLPAVWGDCGLPPDVPNAQPALEGRTSFPEDTVITYKCEESFVKIPGEKDSVICLKGSQWSDIEEFCNRSCEVPTRLNSASLKQPYITQNYFPVGTVVEYECRPGYRREPSLSPKLTCLQNLKWSTAVEFCKKKSCPNPGEIRNGQIDVPGGILFGATISFSCNTGYKLFGSTSSFCLISGSSVQWSDPLPECREIYCPAPPQIDNGIIQGERDHYGYRQSVTYACNKGFTMIGEHSIYCTVNNDEGEWSGPPPECRGKSLTSKVPPTVQKPTTVNVPTTEVSPTSQKTTTKTTTPNAQATRSTPVSRTTKHFHETTPNKGSGTTSGTTRLLSGHTCFTLTGLLGTLVTMGLLT

SEQ ID NO: 2 - DNA, 1146 bp, artificial sequence
  source 1..1146: mol_type = other DNA
atgaccgtcgcgcggccgagcgtgcccgcggcgctgcccctcctcggggagctgccccggctgctgctgctggtgctgttgtgcctgccggccgtgtggggtgactgtggccttcccccagatgtacctaatgcccagccagctttggaaggccgtacaagttttcccgaggatactgtaataacgtacaaatgtgaagaaagctttgtgaaaattcctggcgagaaggactcagtgatctgccttaagggcagtcaatggtcagatattgaagagttctgcaatcgtagctgcgaggtgccaacaaggctaaattctgcatccctcaaacagccttatatcactcagaattattttccagtcggtactgttgtggaatatgagtgccgtccaggttacagaagagaaccttctctatcaccaaaactaacttgccttcagaatttaaaatggtccacagcagtcgaattttgtaaaaagaaatcatgccctaatccgggagaaatacgaaatggtcagattgatgtaccaggtggcatattatttggtgcaaccatctccttctcatgtaacacagggtacaaattatttggctcgacttctagtttttgtcttatttcaggcagctctgtccagtggagtgacccgttgccagagtgcagagaaatttattgtccagcaccaccacaaattgacaatggaataattcaaggggaacgtgaccattatggatatagacagtctgtaacgtatgcatgtaataaaggattcaccatgattggagagcactctatttattgtactgtgaataatgatgaaggagagtggagtggcccaccacctgaatgcagaggaaaatctctaacttccaaggtcccaccaacagttcagaaacctaccacagtaaatgttccaactacagaagtctcaccaacttctcagaaaaccaccacaaaaaccaccacaccaaatgctcaagcaacacggagtacacctgtttccaggacaaccaagcattttcatgaaacaaccccaaataaaggaagtggaaccacttcaggtactacccgtcttctatctgggcacacgtgtttcacgttgacaggtttgcttgggacgctagtaaccatgggcttgctgacttag

SEQ ID NO: 3 - protein, 1231 aa, artificial sequence
MRLLAKIICLMLWAICVAEDCNELPPRRNTEILTGSWSDQTYPEGTQAIYKCRPGYRSLGNVIMVCRKGEWVALNPLRKCQKRPCGHPGDTPFGTFTLTGGNVFEYGVKAVYTCNEGYQLLGEINYRECDTDGWTNDIPICEVVKCLPVTAPENGKIVSSAMEPDREYHFGQAVRFVCNSGYKIEGDEEMHCSDDGFWSKEKPKCVEISCKSPDVINGSPISQKIIYKENERFQYKCNMGYEYSERGDAVCTESGWRPLPSCEEKSCDNPYIPNGDYSPLRIKHRTGDEITYQCRNGFYPATRGNTAKCTSTGWIPAPRCTLKPCDYPDIKHGGLYHENMRRPYFPVAVGKYYSYYCDEHFETPSGSYWDHIHCTQDGWSPAVPCLRKCYFPYLENGYNQNYGRKFVQGKSIDVACHPGYALPKAQTTVTCMENGWSPTPRCIRVKTCSKSSIDIENGFISESQYTYALKEKAKYQCKLGYVTADGETSGSITCGKDGWSAQPTCIKSCDIPVFMNARTKNDFTWFKLNDTLDYECHDGYESNTGSTTGSIVCGYNGWSDLPICYERECELPKIDVHLVPDRKKDQYKVGEVLKFSCKPGFTIVGPNSVQCYHFGLSPDLPICKEQVQSCGPPPELLNGNVKEKTKEEYGHSEVVEYYCNPRFLMKGPNKIQCVDGEWTTLPVCIVEESTCGDIPELEHGWAQLSSPPYYYGDSVEFNCSESFTMIGHRSITCIHGVWTQLPQCVAIDKLKKCKSSNLIILEEHLKNKKEFDHNSNIRYRCRGKEGWIHTVCINGRWDPEVNCSMAQIQLCPPPPQIPNSHNMTTTLNYRDGEKVSVLCQENYLIQEGEEITCKDGRWQSIPLCVEKIPCSQPPQIEHGTINSSRSSQESYAHGTKLSYTCEGGFRISEENETTCYMGKWSSPPQCEGLPCKSPPEISHGVVAHMSDSYQYGEEVTYKCFEGFGIDGPAIAKCLGEKWSHPPSCIKTDCLSLPSFENAIPMGEKKDVYKAGEQVTYTCATYYKMDGASNVTCINSRWTGRPTCRDTSCVNPPTVQNAYIVSRQMSKYPSGERVRYQCRSPYEMFGDEEVMCLNGNWTEPPQCKDSTGKCGPPPPIDNGDITSFPLSVYAPASSVEYQCQNLYQLEGNKRITCRNGQWSEPPKCLHPCVISREIMENYNIALRWTAKQKLYSRTGESVEFVCKRGYRLSSRSHTLRTTCWDGKLEYPTCAKR

SEQ ID NO: 4 - DNA, 3696 bp, artificial sequence
  source 1..3696: mol_type = other DNA
atgagacttctagcaaagattatttgccttatgttatgggctatttgtgtagcagaagattgcaatgaacttcctccaagaagaaatacagaaattctgacaggttcctggtctgaccaaacatatccagaaggcacccaggctatctataaatgccgccctggatatagatctcttggaaatgtaataatggtatgcaggaagggagaatgggttgctcttaatccattaaggaaatgtcagaaaaggccctgtggacatcctggagatactccttttggtacttttacccttacaggaggaaatgtgtttgaatatggtgtaaaagctgtgtatacatgtaatgaggggtatcaattgctaggtgagattaattaccgtgaatgtgacacagatggatggaccaatgatattcctatatgtgaagttgtgaagtgtttaccagtgacagcaccagagaatggaaaaattgtcagtagtgcaatggaaccagatcgggaataccattttggacaagcagtacggtttgtatgtaactcaggctacaagattgaaggagatgaagaaatgcattgttcagacgatggtttttggagtaaagagaaaccaaagtgtgtggaaatttcatgcaaatccccagatgttataaatggatctcctatatctcagaagattatttataaggagaatgaacgatttcaatataaatgtaacatgggttatgaatacagtgaaagaggagatgctgtatgcactgaatctggatggcgtccgttgccttcatgtgaagaaaaatcatgtgataatccttatattccaaatggtgactactcacctttaaggattaaacacagaactggagatgaaatcacgtaccagtgtagaaatggtttttatcctgcaacccggggaaatacagcaaaatgcacaagtactggctggatacctgctccgagatgtaccttgaaaccttgtgattatccagacattaaacatggaggtctatatcatgagaatatgcgtagaccatactttccagtagctgtaggaaaatattactcctattactgtgatgaacattttgagactccgtcaggaagttactgggatcacattcattgcacacaagatggatggtcgccagcagtaccatgcctcagaaaatgttattttccttatttggaaaatggatataatcaaaatcatggaagaaagtttgtacagggtaaatctatagacgttgcctgccatcctggctacgctcttccaaaagcgcagaccacagttacatgtatggagaatggctggtctcctactcccagatgcatccgtgtcaaaacatgttccaaatcaagtatagatattgagaatgggtttatttctgaatctcagtatacatatgccttaaaagaaaaagcgaaatatcaatgcaaactaggatatgtaacagcagatggtgaaacatcaggatcaattacatgtgggaaagatggatggtcagctcaacccacgtgcattaaatcttgtgatatcccagtatttatgaatgccagaactaaaaatgacttcacatggtttaagctgaatgacacattggactatgaatgccatgatggttatgaaagcaatactggaagcaccactggttccatagtgtgtggttacaatggttggtctgatttacccatatgttatgaaagagaatgcgaacttcctaaaatagatgtacacttagttcctgatcgcaagaaagaccagtataaagttggagaggtgttgaaattctcctgcaaaccaggatttacaatagttggacctaattccgttcagtgctaccactttggattgtctcctgacctcccaatatgtaaagagcaagtacaatcatgtggtccacctcctgaactcctcaatgggaatgttaaggaaaaaacgaaagaagaatatggacacagtgaagtggtggaatattattgcaatcctagatttctaatgaagggacctaataaaattcaatgtgttgatggagagtggacaactttaccagtgtgtattgtggaggagagtacctgtggagatatacctgaacttgaacatggctgggcccagctttcttcccctccttattactatggagattcagtggaattcaattgctcagaatcatttacaatgattggacacagatcaattacgtgtattcatggagtatggacccaacttccccagtgtgtggcaatagataaacttaagaagtgcaaatcatcaaatttaattatacttgaggaacatttaaaaaacaagaaggaattcgatcataattctaacataaggtacagatgtagaggaaaagaaggatggatacacacagtctgcataaatggaagatgggatccagaagtgaactgctcaatggcacaaatacaattatgcccacctccacctcagattcccaattctcacaatatgacaaccacactgaattatcgggatggagaaaaagtatctgttctttgccaagaaaattatctaattcaggaaggagaagaaattacatgcaaagatggaagatggcagtcaataccactctgtgttgaaaaaattccatgttcacaaccacctcagatagaacacggaaccattaattcatccaggtcttcacaagaaagttatgcacatgggactaaattgagttatacttgtgagggtggtttcaggatatctgaagaaaatgaaacaacatgctacatgggaaaatggagttctccacctcagtgtgaaggccttccttgtaaatctccacctgagatttctcatggtgttgtagctcacatgtcagacagttatcagtatggagaagaagttacgtacaaatgttttgaaggttttggaattgatgggcctgcaattgcaaaatgcttaggagaaaaatggtctcaccctccatcatgcataaaaacagattgtctcagtttacctagctttgaaaatgccatacccatgggagagaagaaggatgtgtataaggcgggtgagcaagtgacttacacttgtgcaacatattacaaaatggatggagccagtaatgtaacatgcattaatagcagatggacaggaaggccaacatgcagagacacctcctgtgtgaatccgcccacagtacaaaatgcttatatagtgtcgagacagatgagtaaatatccatctggtgagagagtacgttatcaatgtaggagcccttatgaaatgtttggggatgaagaagtgatgtgtttaaatggaaactggacggaaccacctcaatgcaaagattctacaggaaaatgtgggccccctccacctattgacaatggggacattacttcattcccgttgtcagtatatgctccagcttcatcagttgagtaccaatgccagaacttgtatcaacttgagggtaacaagcgaataacatgtagaaatggacaatggtcagaaccaccaaaatgcttacatccgtgtgtaatatcccgagaaattatggaaaattataacatagcattaaggtggacagccaaacagaagctttattcgagaacaggtgaatcagttgaatttgtgtgtaaacggggatatcgtctttcatcacgttctcacacattgcgaacaacatgttgggatgggaaactggagtatccaacttgtgcaaaaagatag

SEQ ID NO: 5 - protein, 449 aa, artificial sequence
MRLLAKIICLMLWAICVAEDCNELPPRRNTEILTGSWSDQTYPEGTQAIYKCRPGYRSLGNVIMVCRKGEWVALNPLRKCQKRPCGHPGDTPFGTFTLTGGNVFEYGVKAVYTCNEGYQLLGEINYRECDTDGWTNDIPICEVVKCLPVTAPENGKIVSSAMEPDREYHFGQAVRFVCNSGYKIEGDEEMHCSDDGFWSKEKPKCVEISCKSPDVINGSPISQKIIYKENERFQYKCNMGYEYSERGDAVCTESGWRPLPSCEEKSCDNPYIPNGDYSPLRIKHRTGDEITYQCRNGFYPATRGNTAKCTSTGWIPAPRCTLKPCDYPDIKHGGLYHENMRRPYFPVAVGKYYSYYCDEHFETPSGSYWDHIHCTQDGWSPAVPCLRKCYFPYLENGYNQNYGRKFVQGKSIDVACHPGYALPKAQTTVTCMENGWSPTPRCIRVSFTL

SEQ ID NO: 6 - DNA, 1350 bp, artificial sequence
  source 1..1350: mol_type = other DNA
atgagacttctagcaaagattatttgccttatgttatgggctatttgtgtagcagaagattgcaatgaacttcctccaagaagaaatacagaaattctgacaggttcctggtctgaccaaacatatccagaaggcacccaggctatctataaatgccgccctggatatagatctcttggaaatgtaataatggtatgcaggaagggagaatgggttgctcttaatccattaaggaaatgtcagaaaaggccctgtggacatcctggagatactccttttggtacttttacccttacaggaggaaatgtgtttgaatatggtgtaaaagctgtgtatacatgtaatgaggggtatcaattgctaggtgagattaattaccgtgaatgtgacacagatggatggaccaatgatattcctatatgtgaagttgtgaagtgtttaccagtgacagcaccagagaatggaaaaattgtcagtagtgcaatggaaccagatcgggaataccattttggacaagcagtacggtttgtatgtaactcaggctacaagattgaaggagatgaagaaatgcattgttcagacgatggtttttggagtaaagagaaaccaaagtgtgtggaaatttcatgcaaatccccagatgttataaatggatctcctatatctcagaagattatttataaggagaatgaacgatttcaatataaatgtaacatgggttatgaatacagtgaaagaggagatgctgtatgcactgaatctggatggcgtccgttgccttcatgtgaagaaaaatcatgtgataatccttatattccaaatggtgactactcacctttaaggattaaacacagaactggagatgaaatcacgtaccagtgtagaaatggtttttatcctgcaacccggggaaatacagcaaaatgcacaagtactggctggatacctgctccgagatgtaccttgaaaccttgtgattatccagacattaaacatggaggtctatatcatgagaatatgcgtagaccatactttccagtagctgtaggaaaatattactcctattactgtgatgaacattttgagactccgtcaggaagttactgggatcacattcattgcacacaagatggatggtcgccagcagtaccatgcctcagaaaatgttattttccttatttggaaaatggatataatcaaaatcatggaagaaagtttgtacagggtaaatctatagacgttgcctgccatcctggctacgctcttccaaaagcgcagaccacagttacatgtatggagaatggctggtctcctactcccagatgcatccgtgtcagctttaccctctga

SEQ ID NO: 7 - protein, 62 aa, artificial sequence
KSCPNPGEIRNGQIDVPGGILFGATISFSCNTGYKLFGSTSSFCLISGSSVQWSDPLPECRE

SEQ ID NO: 8 - protein, 60 aa, artificial sequence
CPNPGEIRNGQIDVPGGILFGATISFSCNTGYKLFGSTSSFCLISGSSVQWSDPLPECRE

SEQ ID NO: 9 - protein, 63 aa, artificial sequence
IYCPAPPQIDNGIIQGERDHYGYRQSVTYACNKGFTMIGEHSIYCTVNNDEGEWSGPPPECRG

SEQ ID NO: 10 - protein, 125 aa, artificial sequence
KSCPNPGEIRNGQIDVPGGILFGATISFSCNTGYKLFGSTSSFCLISGSSVQWSDPLPECREIYCPAPPQIDNGIIQGERDHYGYRQSVTYACNKGFTMIGEHSIYCTVNNDEGEWSGPPPECRG

SEQ ID NO: 11 - protein, 123 aa, artificial sequence
CPNPGEIRNGQIDVPGGILFGATISFSCNTGYKLFGSTSSFCLISGSSVQWSDPLPECREIYCPAPPQIDNGIIQGERDHYGYRQSVTYACNKGFTMIGEHSIYCTVNNDEGEWSGPPPECRG

SEQ ID NO: 12 - protein, 66 aa, artificial sequence
EDCNELPPRRNTEILTGSWSDQTYPEGTQAIYKCRPGYRSLGNVIMVCRKGEWVALNPLRKCQKRP

SEQ ID NO: 13 - protein, 64 aa, artificial sequence
EDCNELPPRRNTEILTGSWSDQTYPEGTQAIYKCRPGYRSLGNVIMVCRKGEWVALNPLRKCQK

SEQ ID NO: 14 - protein, 66 aa, artificial sequence
EDCNELPPRRNTEILTGSWSDQTYPEGTQAIYKCRPGYRSLGNIIMVCRKGEWVALNPLRKCQKRP

SEQ ID NO: 15 - protein, 64 aa, artificial sequence
EDCNELPPRRNTEILTGSWSDQTYPEGTQAIYKCRPGYRSLGNIIMVCRKGEWVALNPLRKCQK

SEQ ID NO: 16 - protein, 7 aa, artificial sequence
GHHHHHH

SEQ ID NO: 17 - protein, 19 aa, artificial sequence
MGWSCIILFLVATATGVHS

SEQ ID NO: 18 - protein, 189 aa, artificial sequence
EDCNELPPRRNTEILTGSWSDQTYPEGTQAIYKCRPGYRSLGNVIMVCRKGEWVALNPLRKCQKRPCPNPGEIRNGQIDVPGGILFGATISFSCNTGYKLFGSTSSFCLISGSSVQWSDPLPECREIYCPAPPQIDNGIIQGERDHYGYRQSVTYACNKGFTMIGEHSIYCTVNNDEGEWSGPPPECRG

SEQ ID NO: 19 - protein, 189 aa, artificial sequence
EDCNELPPRRNTEILTGSWSDQTYPEGTQAIYKCRPGYRSLGNVIMVCRKGEWVALNPLRKCQKKSCPNPGEIRNGQIDVPGGILFGATISFSCNTGYKLFGSTSSFCLISGSSVQWSDPLPECREIYCPAPPQIDNGIIQGERDHYGYRQSVTYACNKGFTMIGEHSIYCTVNNDEGEWSGPPPECRG

SEQ ID NO: 20 - protein, 189 aa, artificial sequence
EDCNELPPRRNTEILTGSWSDQTYPEGTQAIYKCRPGYRSLGNIIMVCRKGEWVALNPLRKCQKKSCPNPGEIRNGQIDVPGGILFGATISFSCNTGYKLFGSTSSFCLISGSSVQWSDPLPECREIYCPAPPQIDNGIIQGERDHYGYRQSVTYACNKGFTMIGEHSIYCTVNNDEGEWSGPPPECRG

SEQ ID NO: 21 - protein, 189 aa, artificial sequence
EDCNELPPRRNTEILTGSWSDQTYPEGTQAIYKCRPGYRSLGNIIMVCRKGEWVALNPLRKCQKRPCPNPGEIRNGQIDVPGGILFGATISFSCNTGYKLFGSTSSFCLISGSSVQWSDPLPECREIYCPAPPQIDNGIIQGERDHYGYRQSVTYACNKGFTMIGEHSIYCTVNNDEGEWSGPPPECRG

SEQ ID NO: 22 - protein, 196 aa, artificial sequence
EDCNELPPRRNTEILTGSWSDQTYPEGTQAIYKCRPGYRSLGNVIMVCRKGEWVALNPLRKCQKRPCPNPGEIRNGQIDVPGGILFGATISFSCNTGYKLFGSTSSFCLISGSSVQWSDPLPECREIYCPAPPQIDNGIIQGERDHYGYRQSVTYACNKGFTMIGEHSIYCTVNNDEGEWSGPPPECRGGHHHHHH

SEQ ID NO: 23 - protein, 196 aa, artificial sequence
EDCNELPPRRNTEILTGSWSDQTYPEGTQAIYKCRPGYRSLGNVIMVCRKGEWVALNPLRKCQKKSCPNPGEIRNGQIDVPGGILFGATISFSCNTGYKLFGSTSSFCLISGSSVQWSDPLPECREIYCPAPPQIDNGIIQGERDHYGYRQSVTYACNKGFTMIGEHSIYCTVNNDEGEWSGPPPECRGGHHHHHH

SEQ ID NO: 24 - protein, 196 aa, artificial sequence
EDCNELPPRRNTEILTGSWSDQTYPEGTQAIYKCRPGYRSLGNIIMVCRKGEWVALNPLRKCQKKSCPNPGEIRNGQIDVPGGILFGATISFSCNTGYKLFGSTSSFCLISGSSVQWSDPLPECREIYCPAPPQIDNGIIQGERDHYGYRQSVTYACNKGFTMIGEHSIYCTVNNDEGEWSGPPPECRGGHHHHHH

SEQ ID NO: 25 - protein, 196 aa, artificial sequence
EDCNELPPRRNTEILTGSWSDQTYPEGTQAIYKCRPGYRSLGNIIMVCRKGEWVALNPLRKCQKRPCPNPGEIRNGQIDVPGGILFGATISFSCNTGYKLFGSTSSFCLISGSSVQWSDPLPECREIYCPAPPQIDNGIIQGERDHYGYRQSVTYACNKGFTMIGEHSIYCTVNNDEGEWSGPPPECRGGHHHHHH

SEQ ID NO: 26 - protein, 215 aa, artificial sequence
MGWSCIILFLVATATGVHSEDCNELPPRRNTEILTGSWSDQTYPEGTQAIYKCRPGYRSLGNVIMVCRKGEWVALNPLRKCQKRPCPNPGEIRNGQIDVPGGILFGATISFSCNTGYKLFGSTSSFCLISGSSVQWSDPLPECREIYCPAPPQIDNGIIQGERDHYGYRQSVTYACNKGFTMIGEHSIYCTVNNDEGEWSGPPPECRGGHHHHHH

SEQ ID NO: 27 - protein, 215 aa, artificial sequence
MGWSCIILFLVATATGVHSEDCNELPPRRNTEILTGSWSDQTYPEGTQAIYKCRPGYRSLGNVIMVCRKGEWVALNPLRKCQKKSCPNPGEIRNGQIDVPGGILFGATISFSCNTGYKLFGSTSSFCLISGSSVQWSDPLPECREIYCPAPPQIDNGIIQGERDHYGYRQSVTYACNKGFTMIGEHSIYCTVNNDEGEWSGPPPECRGGHHHHHH

SEQ ID NO: 28 - protein, 215 aa, artificial sequence
MGWSCIILFLVATATGVHSEDCNELPPRRNTEILTGSWSDQTYPEGTQAIYKCRPGYRSLGNIIMVCRKGEWVALNPLRKCQKKSCPNPGEIRNGQIDVPGGILFGATISFSCNTGYKLFGSTSSFCLISGSSVQWSDPLPECREIYCPAPPQIDNGIIQGERDHYGYRQSVTYACNKGFTMIGEHSIYCTVNNDEGEWSGPPPECRGGHHHHHH

SEQ ID NO: 29 - protein, 215 aa, artificial sequence
MGWSCIILFLVATATGVHSEDCNELPPRRNTEILTGSWSDQTYPEGTQAIYKCRPGYRSLGNIIMVCRKGEWVALNPLRKCQKRPCPNPGEIRNGQIDVPGGILFGATISFSCNTGYKLFGSTSSFCLISGSSVQWSDPLPECREIYCPAPPQIDNGIIQGERDHYGYRQSVTYACNKGFTMIGEHSIYCTVNNDEGEWSGPPPECRGGHHHHHH

SEQ ID NO: 30 - protein, 208 aa, artificial sequence
MGWSCIILFLVATATGVHSEDCNELPPRRNTEILTGSWSDQTYPEGTQAIYKCRPGYRSLGNVIMVCRKGEWVALNPLRKCQKRPCPNPGEIRNGQIDVPGGILFGATISFSCNTGYKLFGSTSSFCLISGSSVQWSDPLPECREIYCPAPPQIDNGIIQGERDHYGYRQSVTYACNKGFTMIGEHSIYCTVNNDEGEWSGPPPECRG

SEQ ID NO: 31 - protein, 208 aa, artificial sequence
MGWSCIILFLVATATGVHSEDCNELPPRRNTEILTGSWSDQTYPEGTQAIYKCRPGYRSLGNVIMVCRKGEWVALNPLRKCQKKSCPNPGEIRNGQIDVPGGILFGATISFSCNTGYKLFGSTSSFCLISGSSVQWSDPLPECREIYCPAPPQIDNGIIQGERDHYGYRQSVTYACNKGFTMIGEHSIYCTVNNDEGEWSGPPPECRG

SEQ ID NO: 32 - protein, 208 aa, artificial sequence
MGWSCIILFLVATATGVHSEDCNELPPRRNTEILTGSWSDQTYPEGTQAIYKCRPGYRSLGNIIMVCRKGEWVALNPLRKCQKKSCPNPGEIRNGQIDVPGGILFGATISFSCNTGYKLFGSTSSFCLISGSSVQWSDPLPECREIYCPAPPQIDNGIIQGERDHYGYRQSVTYACNKGFTMIGEHSIYCTVNNDEGEWSGPPPECRG

SEQ ID NO: 33 - protein, 208 aa, artificial sequence
MGWSCIILFLVATATGVHSEDCNELPPRRNTEILTGSWSDQTYPEGTQAIYKCRPGYRSLGNIIMVCRKGEWVALNPLRKCQKRPCPNPGEIRNGQIDVPGGILFGATISFSCNTGYKLFGSTSSFCLISGSSVQWSDPLPECREIYCPAPPQIDNGIIQGERDHYGYRQSVTYACNKGFTMIGEHSIYCTVNNDEGEWSGPPPECRG

SEQ ID NO: 34 - protein, 199 aa, artificial sequence
QCNAPEWLPFARPTNLTDEFEFPIGTYLKYECRPGYYGRPFSIICLKNSVWTGAKDRCRRKSCRNPPDPVNGMVHVIKDIQFGSQIKYSCTKGYRLIGSSSATCIISGNTVIWDNETPICDRIPCGLPPTITNGDFISTNRENFHYGSVVTYRCNPGSGGRKVFELVGEPSIYCTSNDDQVGIWSGPAPQCIGHHHHHH

SEQ ID NO: 35 - protein, 196 aa, artificial sequence
SCEVPTRLNSASLKQPYITQNYFPVGTVVEYECRPGYRREPSLSPKLTCLQNLKWSTAVEFCKKKSCPNPGEIRNGQIDVPGGILFGATISFSCNTGYKLFGSTSSFCLISGSSVQWSDPLPECREIYCPAPPQIDNGIIQGERDHYGYRQSVTYACNKGFTMIGEHSIYCTVNNDEGEWSGPPPECRGGHHHHHH

SEQ ID NO: 36 - protein, 313 aa, artificial sequence
EDCNELPPRRNTEILTGSWSDQTYPEGTQAIYKCRPGYRSLGNIIMVCRKGEWVALNPLRKCQKRPCGHPGDTPFGTFTLTGGNVFEYGVKAVYTCNEGYQLLGEINYRECDTDGWTNDIPICEVVKCLPVTAPENGKIVSSAMEPDREYHFGQAVRFVCNSGYKIEGDEEMHCSDDGFWSKEKPKCVEISCKSPDVINGSPISQKIIYKENERFQYKCNMGYEYSERGDAVCTESGWRPLPSCEEKSCDNPYIPNGDYSPLRIKHRTGDEITYQCRNGFYPATRGNTAKCTSTGWIPAPRCTLKPGHHHHHH

SEQ ID NO: 37 - protein, 193 aa, artificial sequence
GHCQAPDHFLFAKLKTQTNASDFPIGTSLKYECRPEYYGRPFSITCLDNLVWSSPKDVCKRKSCPNPGEIRNGQIDVPGGILFGATISFSCNTGYKLFGSTSSFCLISGSSVQWSDPLPECREIYCPAPPQIDNGIIQGERDHYGYRQSVTYACNKGFTMIGEHSIYCTVNNDEGEWSGPPPECRGGHHHHHH

SEQ ID NO: 38 - protein, 1658 aa, artificial sequence
QEQTYVISAPKIFRVGASENIVIQVYGYTEAFDATISIKSYPDKKFSYSSGHVHLSSENKFQNSAILTIQPKQLPGGQNPVSYVYLEVVSKHFSKSKRMPITYDNGFLFIHTDKPVYTPDQSVKVRVYSLNDDLKPAKRETVLTFIDPEGSEVDMVEEIDHIGIISFPDFKIPSNPRYGMWTIKAKYKEDFSTTGTAYFEVKEYVLPHFSVSIEPEYNFIGYKNFKNFEITIKARYFYNKVVTEADVYITFGIREDLKDDQKEMMQTAMQNTMLINGIAQVTFDSETAVKELSYYSLEDLNNKYLYIAVTVIESTGGFSEEAEIPGIKYVLSPYKLNLVATPLFLKPGIPYPIKVQVKDSLDQLVGGVPVTLNAQTIDVNQETSDLDPSKSVTRVDDGVASFVLNLPSGVTVLEFNVKTDAPDLPEENQAREGYRAIAYSSLSQSYLYIDWTDNHKALLVGEHLNIIVTPKSPYIDKITHYNYLILSKGKIIHFGTREKFSDASYQSINIPVTQNMVPSSRLLVYYIVTGEQTAELVSDSVWLNIEEKCGNQLQVHLSPDADAYSPGQTVSLNMATGMDSWVALAAVDSAVYGVQRGAKKPLERVFQFLEKSDLGCGAGGGLNNANVFHLAGLTFLTNANADDSQENDEPCKEILRPRRTLQKKIEEIAAKYKHSVVKKCCYDGACVNNDETCEQRAARISLGPRCIKAFTECCVVASQLRANISHKDMQLGRLHMKTLLPVSKPEIRSYFPESWLWEVHLVPRRKQLQFALPDSLTTWEIQGVGISNTGICVADTVKAKVFKDVFLEMNIPYSVVRGEQIQLKGTVYNYRTSGMQFCVKMSAVEGICTSESPVIDHQGTKSSKCVRQKVEGSSSHLVTFTVLPLEIGLHNINFSLETWFGKEILVKTLRVVPEGVKRESYSGVTLDPRGIYGTISRRKEFPYRIPLDLVPKTEIKRILSVKGLLVGEILSAVLSQEGINILTHLPKGSAEAELMSVVPVFYVFHYLETGNHWNIFHSDPLIEKQKLKKKLKEGMLSIMSYRNADYSYSVWKGGSASTWLTAFALRVLGQVNKYVEQNQNSICNSLLWLVENYQLDNGSFKENSQYQPIKLQGTLPVEARENSLYLTAFTVIGIRKAFDICPLVKIDTALIKADNFLLENTLPAQSTFTLAISAYALSLGDKTHPQFRSIVSALKREALVKGNPPIYRFWKDNLQHKDSSVPNTGTARMVETTAYALLTSLNLKDINYVNPVIKWLSEEQRYGGGFYSTQDTINAIEGLTEYSLLVKQLRLSMDIDVSYKHKGALHNYKMTDKNFLGRPVEVLLNDDLIVSTGFGSGLATVHVTTVVHKTSTSEEVCSFYLKIDTQDIEASHYRGYGNSDYKRIVACASYKPSREESSSGSSHAVMDISLPTGISANEEDLKALVEGVDQLFTDYQIKDGHVILQLNSIPSSDFLCVRFRIFELFEVGFLSPATFTVYEYHRPDKQCTMFYSTSNIKIQKVCEGAACKCVEADCGQMQEELDLTISAETRKQTACKPEIAYAYKVSITSITVENVFVKYKATLLDIYKTGEAVAEKDSEITFIKKVTCTNAELVKGRQYLIMGKEALQIKYNFSFRYIYPLDSLTWIEYWPRDTTCSSCQAFLANLDEFAEDIFLNGC

SEQ ID NO: 39 - protein, 122 aa, artificial sequence
QVQLVQSGAEVKKPGASVKVSCKASGYTFTNYGMNWVRQAPGQGLEWMGWINTYTGEPTYADDFKGRFTFTLDTSTSTAYLELSSLRSEDTAVYYCARTKVPHYFAYAMDYWGQGTLVTVSS

SEQ ID NO: 40 - protein, 7 aa, artificial sequence
GYTFTNY

SEQ ID NO: 41 - protein, 6 aa, artificial sequence
NTYTGE

SEQ ID NO: 42 - protein, 13 aa, artificial sequence
TKVPHYFAYAMDY

SEQ ID NO: 43 - protein, 327 aa, artificial sequence
ASTKGPSVFPLAPCSRSTSESTAALGCLVKDYFPEPVTVSWNSGALTSGVHTFPAVLQSSGLYSLSSVVTVPSSSLGTKTYTCNVDHKPSNTKVDKRVESKYGPPCPPCPAPEFLGGPSVFLFPPKPKDTLMISRTPEVTCVVVDVSQEDPEVQFNWYVDGVEVHNAKTKPREEQFNSTYRVVSVLTVLHQDWLNGKEYKCKVSNKGLPSSIEKTISKAKGQPREPQVYTLPPSQEEMTKNQVSLTCLVKGFYPSDIAVEWESNGQPENNYKTTPPVLDSDGSFFLYSRLTVDKSRWQEGNVFSCSVLHEALHAHYTQKSLSLSLGK

SEQ ID NO: 44 - protein, 449 aa, artificial sequence
QVQLVQSGAEVKKPGASVKVSCKASGYTFTNYGMNWVRQAPGQGLEWMGWINTYTGEPTYADDFKGRFTFTLDTSTSTAYLELSSLRSEDTAVYYCARTKVPHYFAYAMDYWGQGTLVTVSSASTKGPSVFPLAPCSRSTSESTAALGCLVKDYFPEPVTVSWNSGALTSGVHTFPAVLQSSGLYSLSSVVTVPSSSLGTKTYTCNVDHKPSNTKVDKRVESKYGPPCPPCPAPEFLGGPSVFLFPPKPKDTLMISRTPEVTCVVVDVSQEDPEVQFNWYVDGVEVHNAKTKPREEQFNSTYRVVSVLTVLHQDWLNGKEYKCKVSNKGLPSSIEKTISKAKGQPREPQVYTLPPSQEEMTKNQVSLTCLVKGFYPSDIAVEWESNGQPENNYKTTPPVLDSDGSFFLYSRLTVDKSRWQEGNVFSCSVLHEALHAHYTQKSLSLSLGK

SEQ ID NO: 45 - protein, 111 aa, artificial sequence
DIVLTQSPSSLSASVGDRVTITCKASQSVDYHGDSYLNWYQQKPGKPPKLLIYAASNLESGIPSRFSGSGSGTDFTLTISSLQPEDFATYYCQQSNEDPSTFGGGTKLEIK

SEQ ID NO: 46 - protein, 15 aa, artificial sequence
KASQSVDYHGDSYLN

SEQ ID NO: 47 - protein, 7 aa, artificial sequence
AASNLES

SEQ ID NO: 48 - protein, 9 aa, artificial sequence
QQSNEDPST

SEQ ID NO: 49 - protein, 107 aa, artificial sequence [sequence omitted]

SEQ ID NO: 50 - protein, 218 aa, artificial sequence
DIVLTQSPSSLSASVGDRVTITCKASQSVDYHGDSYLNWYQQKPGKPPKLLIYAASNLESGIPSRFSGSGSGTDFTLTISSLQPEDFATYYCQQSNEDPSTFGGGTKLEIKRTVAAPSVFIFPPSDEQLKSGTASVVCLLNNFYPREAKVQWKVDNALQSGNSQESVTEQDSKDSTYSLSSTLTLSKADYEKHKVYACEVTHQGLSSPVTKSFNRGEC

SEQ ID NO: 51 - protein, 198 aa, artificial sequence
EDCNELPPRRNTEILTGSWSDQTYPEGTQAIYKCRPGYRSLGNIIMVCRKGEWVALNPLRKCQKRPCGHPGDTPFGTFTLTGGNVFEYGVKAVYTCNEGYQLLGEINYRECDTDGWTNDIPICEVVKCLPVTAPENGKIVSSAMEPDREYHFGQAVRFVCNSGYKIEGDEEMHCSDDGFWSKEKPKCVEISGHHHHHH

SEQ ID NO: 52 - protein, 260 aa, artificial sequence
DCGLPPDVPNAQPALEGRTSFPEDTVITYKCEESFVKIPGEKDSVICLKGSQWSDIEEFCNRSCEVPTRLNSASLKQPYITQNYFPVGTVVEYECRPGYRREPSLSPKLTCLQNLKWSTAVEFCKKKSCPNPGEIRNGQIDVPGGILFGATISFSCNTGYKLFGSTSSFCLISGSSVQWSDPLPECREIYCPAPPQIDNGIIQGERDHYGYRQSVTYACNKGFTMIGEHSIYCTVNNDEGEWSGPPPECRGKSGHHHHHH

SEQ ID NO: 53 - protein, 198 aa, artificial sequence
EDCNELPPRRNTEILTGSWSDQTYPEGTQAIYKCRPGYRSLGNIIMVCRKGEWVAENPSRKCQKKSCPNPGEIRNGQIDVPDGILFGATISFSCNTGYKLFGSTSSFCLTSGSSVQWSDPLPECREIYCPAPPQIDNGIIQGERDHYGYRQSVTYACNKGFTMIGEHSIYCTVNNDEGEWSGPPPECRGKSGHHHHHH

SEQ ID NO: 54 - protein, 198 aa, artificial sequence
EDCNELPPRRNTEILTGSWSDQTYPEGTQAIYKCRPGYRSLGNIIMVCRKGEWVAENPDRKCQKKSCPNPGEIRNGQIDVPDGILFGATISFSCNTGYKLFGSTSSFCLTSGSSVQWSDPLPECREIYCPAPPQIDNGIIQGERDHYGYRQSVTYACNKGFTMIGEHSIYCTVNNDEGEWSGPPPECRGKSGHHHHHH

SEQ ID NO: 55 - protein, 641 aa, artificial sequence
QVQLVQSGAEVKKPGASVKVSCKASGYTFTNYGMNWVRQAPGQGLEWMGWINTYTGEPTYADDFKGRFTFTLDTSTSTAYLELSSLRSEDTAVYYCARTKVPHYFAYAMDYWGQGTLVTVSSASTKGPSVFPLAPCSRSTSESTAALGCLVKDYFPEPVTVSWNSGALTSGVHTFPAVLQSSGLYSLSSVVTVPSSSLGTKTYTCNVDHKPSNTKVDKRVESKYGPPCPPCPAPEFLGGPSVFLFPPKPKDTLMISRTPEVTCVVVDVSQEDPEVQFNWYVDGVEVHNAKTKPREEQFNSTYRVVSVLTVLHQDWLNGKEYKCKVSNKGLPSSIEKTISKAKGQPREPQVYTLPPSQEEMTKNQVSLTCLVKGFYPSDIAVEWESNGQPENNYKTTPPVLDSDGSFFLYSRLTVDKSRWQEGNVFSCSVLHEALHAHYTQKSLSLSLGKGSGEDCNELPPRRNTEILTGSWSDQTYPEGTQAIYKCRPGYRSLGNIIMVCRKGEWVALNPLRKCQKKSCPNPGEIRNGQIDVPGGILFGATISFSCNTGYKLFGSTSSFCLISGSSVQWSDPLPECREIYCPAPPQIDNGIIQGERDHYGYRQSVTYACNKGFTMIGEHSIYCTVNNDEGEWSGPPPECRG

SEQ ID NO: 56 - protein, 198 aa, artificial sequence
EDCNELPPRRNTEILTGSWSDQTYPEGTQAIYKCRPGYRSLGNIIMVCRKGEWVALNPLRKCQKKSCPNPGEIRNGQIDVPGGILFGATISFSCNTGYKLFGSTSSFCLISGSSVQWSDPLPECREIYCPAPPQIDNGIIQGERDHYGYRQSVTYACNKGFTMIGEHSIYCTVNNDEGEWSGPPPECRGKSGHHHHHH

SEQ ID NO: 57 - protein, 198 aa, artificial sequence
EDCNELPPRRNTEILTGSWSDQTYPEGTQAIYKCRPGYRSLGNIIMVCRKGEWVAENPLRKCQKKSCPNPGEIRNGQIDVPGGILFGATISFSCNTGYKLFGSTSSFCLISGSSVQWSDPLPECREIYCPAPPQIDNGIIQGERDHYGYRQSVTYACNKGFTMIGEHSIYCTVNNDEGEWSGPPPECRGKSGHHHHHH

SEQ ID NO: 58 - protein, 198 aa, artificial sequence
EDCNELPPRRNTEILTGSWSDQTYPEGTQAIYKCRPGYRSLGNIIMVCRKGEWVALNPDRKCQKKSCPNPGEIRNGQIDVPGGILFGATISFSCNTGYKLFGSTSSFCLISGSSVQWSDPLPECREIYCPAPPQIDNGIIQGERDHYGYRQSVTYACNKGFTMIGEHSIYCTVNNDEGEWSGPPPECRGKSGHHHHHH

SEQ ID NO: 59 - protein, 217 aa, artificial sequence
APEFLGGPSVFLFPPKPKDTLMISRTPEVTCVVVDVSQEDPEVQFNWYVDGVEVHNAKTKPREEQFNSTYRVVSVLTVLHQDWLNGKEYKCKVSNKGLPSSIEKTISKAKGQPREPQVYTLPPSQEEMTKNQVSLTCLVKGFYPSDIAVEWESNGQPENNYKTTPPVLDSDGSFFLYSRLTVDKSRWQEGNVFSCSVLHEALHAHYTQKSLSLSLGK

SEQ ID NO: 60 - protein, 191 aa, artificial sequence
EDCNELPPRRNTEILTGSWSDQTYPEGTQAIYKCRPGYRSLGNIIMVCRKGEWVALNPLRKCQKKSCPNPGEIRNGQIDVPGGILFGATISFSCNTGYKLFGSTSSFCLISGSSVQWSDPLPECREIYCPAPPQIDNGIIQGERDHYGYRQSVTYACNKGFTMIGEHSIYCTVNNDEGEWSGPPPECRGKS

SEQ ID NO: 61 - protein, 643 aa, artificial sequence
QVQLVQSGAEVKKPGASVKVSCKASGYTFTNYGMNWVRQAPGQGLEWMGWINTYTGEPTYADDFKGRFTFTLDTSTSTAYLELSSLRSEDTAVYYCARTKVPHYFAYAMDYWGQGTLVTVSSASTKGPSVFPLAPCSRSTSESTAALGCLVKDYFPEPVTVSWNSGALTSGVHTFPAVLQSSGLYSLSSVVTVPSSSLGTKTYTCNVDHKPSNTKVDKRVESKYGPPCPPCPAPEFLGGPSVFLFPPKPKDTLMISRTPEVTCVVVDVSQEDPEVQFNWYVDGVEVHNAKTKPREEQFNSTYRVVSVLTVLHQDWLNGKEYKCKVSNKGLPSSIEKTISKAKGQPREPQVYTLPPSQEEMTKNQVSLTCLVKGFYPSDIAVEWESNGQPENNYKTTPPVLDSDGSFFLYSRLTVDKSRWQEGNVFSCSVLHEALHAHYTQKSLSLSLGKGSGEDCNELPPRRNTEILTGSWSDQTYPEGTQAIYKCRPGYRSLGNIIMVCRKGEWVALNPLRKCQKKSCPNPGEIRNGQIDVPGGILFGATISFSCNTGYKLFGSTSSFCLISGSSVQWSDPLPECREIYCPAPPQIDNGIIQGERDHYGYRQSVTYACNKGFTMIGEHSIYCTVNNDEGEWSGPPPECRGKS

SEQ ID NO: 62 - protein, 191 aa, artificial sequence
EDCNELPPRRNTEILTGSWSDQTYPEGTQAIYKCRPGYRSLGNIIMVCRKGEWVAENPLRKCQKKSCPNPGEIRNGQIDVPGGILFGATISFSCNTGYKLFGSTSSFCLISGSSVQWSDPLPECREIYCPAPPQIDNGIIQGERDHYGYRQSVTYACNKGFTMIGEHSIYCTVNNDEGEWSGPPPECRGKS

SEQ ID NO: 63 - protein, 643 aa, artificial sequence
QVQLVQSGAEVKKPGASVKVSCKASGYTFTNYGMNWVRQAPGQGLEWMGWINTYTGEPTYADDFKGRFTFTLDTSTSTAYLELSSLRSEDTAVYYCARTKVPHYFAYAMDYWGQGTLVTVSSASTKGPSVFPLAPCSRSTSESTAALGCLVKDYFPEPVTVSWNSGALTSGVHTFPAVLQSSGLYSLSSVVTVPSSSLGTKTYTCNVDHKPSNTKVDKRVESKYGPPCPPCPAPEFLGGPSVFLFPPKPKDTLMISRTPEVTCVVVDVSQEDPEVQFNWYVDGVEVHNAKTKPREEQFNSTYRVVSVLTVLHQDWLNGKEYKCKVSNKGLPSSIEKTISKAKGQPREPQVYTLPPSQEEMTKNQVSLTCLVKGFYPSDIAVEWESNGQPENNYKTTPPVLDSDGSFFLYSRLTVDKSRWQEGNVFSCSVLHEALHAHYTQKSLSLSLGKGSGEDCNELPPRRNTEILTGSWSDQTYPEGTQAIYKCRPGYRSLGNIIMVCRKGEWVAENPLRKCQKKSCPNPGEIRNGQIDVPGGILFGATISFSCNTGYKLFGSTSSFCLISGSSVQWSDPLPECREIYCPAPPQIDNGIIQGERDHYGYRQSVTYACNKGFTMIGEHSIYCTVNNDEGEWSGPPPECRGKS

SEQ ID NO: 64 - protein, 191 aa, artificial sequence
EDCNELPPRRNTEILTGSWSDQTYPEGTQAIYKCRPGYRSLGNIIMVCRKGEWVALNPDRKCQKKSCPNPGEIRNGQIDVPGGILFGATISFSCNTGYKLFGSTSSFCLISGSSVQWSDPLPECREIYCPAPPQIDNGIIQGERDHYGYRQSVTYACNKGFTMIGEHSIYCTVNNDEGEWSGPPPECRGKS

SEQ ID NO: 65 - protein, 643 aa, artificial sequence
QVQLVQSGAEVKKPGASVKVSCKASGYTFTNYGMNWVRQAPGQGLEWMGWINTYTGEPTYADDFKGRFTFTLDTSTSTAYLELSSLRSEDTAVYYCARTKVPHYFAYAMDYWGQGTLVTVSSASTKGPSVFPLAPCSRSTSESTAALGCLVKDYFPEPVTVSWNSGALTSGVHTFPAVLQSSGLYSLSSVVTVPSSSLGTKTYTCNVDHKPSNTKVDKRVESKYGPPCPPCPAPEFLGGPSVFLFPPKPKDTLMISRTPEVTCVVVDVSQEDPEVQFNWYVDGVEVHNAKTKPREEQFNSTYRVVSVLTVLHQDWLNGKEYKCKVSNKGLPSSIEKTISKAKGQPREPQVYTLPPSQEEMTKNQVSLTCLVKGFYPSDIAVEWESNGQPENNYKTTPPVLDSDGSFFLYSRLTVDKSRWQEGNVFSCSVLHEALHAHYTQKSLSLSLGKGSGEDCNELPPRRNTEILTGSWSDQTYPEGTQAIYKCRPGYRSLGNIIMVCRKGEWVALNPDRKCQKKSCPNPGEIRNGQIDVPGGILFGATISFSCNTGYKLFGSTSSFCLISGSSVQWSDPLPECREIYCPAPPQIDNGIIQGERDHYGYRQSVTYACNKGFTMIGEHSIYCTVNNDEGEWSGPPPECRGKS

SEQ ID NO: 66 - protein, 191 aa, artificial sequence
EDCNELPPRRNTEILTGSWSDQTYPEGTQAIYKCRPGYRSLGNIIMVCRKGEWVALNPSRKCQKKSCPNPGEIRNGQIDVPGGILFGATISFSCNTGYKLFGSTSSFCLISGSSVQWSDPLPECREIYCPAPPQIDNGIIQGERDHYGYRQSVTYACNKGFTMIGEHSIYCTVNNDEGEWSGPPPECRGKS

SEQ ID NO: 67 - protein, 643 aa, artificial sequence
QVQLVQSGAEVKKPGASVKVSCKASGYTFTNYGMNWVRQAPGQGLEWMGWINTYTGEPTYADDFKGRFTFTLDTSTSTAYLELSSLRSEDTAVYYCARTKVPHYFAYAMDYWGQGTLVTVSSASTKGPSVFPLAPCSRSTSESTAALGCLVKDYFPEPVTVSWNSGALTSGVHTFPAVLQSSGLYSLSSVVTVPSSSLGTKTYTCNVDHKPSNTKVDKRVESKYGPPCPPCPAPEFLGGPSVFLFPPKPKDTLMISRTPEVTCVVVDVSQEDPEVQFNWYVDGVEVHNAKTKPREEQFNSTYRVVSVLTVLHQDWLNGKEYKCKVSNKGLPSSIEKTISKAKGQPREPQVYTLPPSQEEMTKNQVSLTCLVKGFYPSDIAVEWESNGQPENNYKTTPPVLDSDGSFFLYSRLTVDKSRWQEGNVFSCSVLHEALHAHYTQKSLSLSLGKGSGEDCNELPPRRNTEILTGSWSDQTYPEGTQAIYKCRPGYRSLGNIIMVCRKGEWVALNPSRKCQKKSCPNPGEIRNGQIDVPGGILFGATISFSCNTGYKLFGSTSSFCLISGSSVQWSDPLPECREIYCPAPPQIDNGIIQGERDHYGYRQSVTYACNKGFTMIGEHSIYCTVNNDEGEWSGPPPECRGKS

SEQ ID NO: 68 - protein, 191 aa, artificial sequence
EDCNELPPRRNTEILTGSWSDQTYPEGTQAIYKCRPGYRSLGNIIMVCRKGEWVALNPLRKCQKKSCPNPGEIRNGQIDVPDGILFGATISFSCNTGYKLFGSTSSFCLISGSSVQWSDPLPECREIYCPAPPQIDNGIIQGERDHYGYRQSVTYACNKGFTMIGEHSIYCTVNNDEGEWSGPPPECRGKS

SEQ ID NO: 69 - protein, 643 aa, artificial sequence
QVQLVQSGAEVKKPGASVKVSCKASGYTFTNYGMNWVRQAPGQGLEWMGWINTYTGEPTYADDFKGRFTFTLDTSTSTAYLELSSLRSEDTAVYYCARTKVPHYFAYAMDYWGQGTLVTVSSASTKGPSVFPLAPCSRSTSESTAALGCLVKDYFPEPVTVSWNSGALTSGVHTFPAVLQSSGLYSLSSVVTVPSSSLGTKTYTCNVDHKPSNTKVDKRVESKYGPPCPPCPAPEFLGGPSVFLFPPKPKDTLMISRTPEVTCVVVDVSQEDPEVQFNWYVDGVEVHNAKTKPREEQFNSTYRVVSVLTVLHQDWLNGKEYKCKVSNKGLPSSIEKTISKAKGQPREPQVYTLPPSQEEMTKNQVSLTCLVKGFYPSDIAVEWESNGQPENNYKTTPPVLDSDGSFFLYSRLTVDKSRWQEGNVFSCSVLHEALHAHYTQKSLSLSLGKGSGEDCNELPPRRNTEILTGSWSDQTYPEGTQAIYKCRPGYRSLGNIIMVCRKGEWVALNPLRKCQKKSCPNPGEIRNGQIDVPDGILFGATISFSCNTGYKLFGSTSSFCLISGSSVQWSDPLPECREIYCPAPPQIDNGIIQGERDHYGYRQSVTYACNKGFTMIGEHSIYCTVNNDEGEWSGPPPECRGKS

SEQ ID NO: 70 - protein, 191 aa, artificial sequence
EDCNELPPRRNTEILTGSWSDQTYPEGTQAIYKCRPGYRSLGNIIMVCRKGEWVALNPLRKCQKKSCPNPGEIRNGQIDVPGGILYGATISFSCNTGYKLFGSTSSFCLISGSSVQWSDPLPECREIYCPAPPQIDNGIIQGERDHYGYRQSVTYACNKGFTMIGEHSIYCTVNNDEGEWSGPPPECRGKS

SEQ ID NO: 71 - protein, 643 aa, artificial sequence
QVQLVQSGAEVKKPGASVKVSCKASGYTFTNYGMNWVRQAPGQGLEWMGWINTYTGEPTYADDFKGRFTFTLDTSTSTAYLELSSLRSEDTAVYYCARTKVPHYFAYAMDYWGQGTLVTVSSASTKGPSVFPLAPCSRSTSESTAALGCLVKDYFPEPVTVSWNSGALTSGVHTFPAVLQSSGLYSLSSVVTVPSSSLGTKTYTCNVDHKPSNTKVDKRVESKYGPPCPPCPAPEFLGGPSVFLFPPKPKDTLMISRTPEVTCVVVDVSQEDPEVQFNWYVDGVEVHNAKTKPREEQFNSTYRVVSVLTVLHQDWLNGKEYKCKVSNKGLPSSIEKTISKAKGQPREPQVYTLPPSQEEMTKNQVSLTCLVKGFYPSDIAVEWESNGQPENNYKTTPPVLDSDGSFFLYSRLTVDKSRWQEGNVFSCSVLHEALHAHYTQKSLSLSLGKGSGEDCNELPPRRNTEILTGSWSDQTYPEGTQAIYKCRPGYRSLGNIIMVCRKGEWVALNPLRKCQKKSCPNPGEIRNGQIDVPGGILYGATISFSCNTGYKLFGSTSSFCLISGSSVQWSDPLPECREIYCPAPPQIDNGIIQGERDHYGYRQSVTYACNKGFTMIGEHSIYCTVNNDEGEWSGPPPECRGKS

SEQ ID NO: 72 - protein, 191 aa, artificial sequence
EDCNELPPRRNTEILTGSWSDQTYPEGTQAIYKCRPGYRSLGNIIMVCRKGEWVALNPLRKCQKKSCPNPGEIRNGQIDVPGGILFGATISFSCNTGYKLFGSTSSECLISGSSVQWSDPLPECREIYCPAPPQIDNGIIQGERDHYGYRQSVTYACNKGFTMIGEHSIYCTVNNDEGEWSGPPPECRGKS

SEQ ID NO: 73 - protein, 643 aa, artificial sequence
QVQLVQSGAEVKKPGASVKVSCKASGYTFTNYGMNWVRQAPGQGLEWMGWINTYTGEPTYADDFKGRFTFTLDTSTSTAYLELSSLRSEDTAVYYCARTKVPHYFAYAMDYWGQGTLVTVSSASTKGPSVFPLAPCSRSTSESTAALGCLVKDYFPEPVTVSWNSGALTSGVHTFPAVLQSSGLYSLSSVVTVPSSSLGTKTYTCNVDHKPSNTKVDKRVESKYGPPCPPCPAPEFLGGPSVFLFPPKPKDTLMISRTPEVTCVVVDVSQEDPEVQFNWYVDGVEVHNAKTKPREEQFNSTYRVVSVLTVLHQDWLNGKEYKCKVSNKGLPSSIEKTISKAKGQPREPQVYTLPPSQEEMTKNQVSLTCLVKGFYPSDIAVEWESNGQPENNYKTTPPVLDSDGSFFLYSRLTVDKSRWQEGNVFSCSVLHEALHAHYTQKSLSLSLGKGSGEDCNELPPRRNTEILTGSWSDQTYPEGTQAIYKCRPGYRSLGNIIMVCRKGEWVALNPLRKCQKKSCPNPGEIRNGQIDVPGGILFGATISFSCNTGYKLFGSTSSECLISGSSVQWSDPLPECREIYCPAPPQIDNGIIQGERDHYGYRQSVTYACNKGFTMIGEHSIYCTVNNDEGEWSGPPPECRGKS

SEQ ID NO: 74 - protein, 191 aa, artificial sequence
EDCNELPPRRNTEILTGSWSDQTYPEGTQAIYKCRPGYRSLGNIIMVCRKGEWVALNPLRKCQKKSCPNPGEIRNGQIDVPGGILFGATISFSCNTGYKLFGSTSSFCDISGSSVQWSDPLPECREIYCPAPPQIDNGIIQGERDHYGYRQSVTYACNKGFTMIGEHSIYCTVNNDEGEWSGPPPECRGKS

SEQ ID NO: 75 - protein, 643 aa, artificial sequence
QVQLVQSGAEVKKPGASVKVSCKASGYTFTNYGMNWVRQAPGQGLEWMGWINTYTGEPTYADDFKGRFTFTLDTSTSTAYLELSSLRSEDTAVYYCARTKVPHYFAYAMDYWGQGTLVTVSSASTKGPSVFPLAPCSRSTSESTAALGCLVKDYFPEPVTVSWNSGALTSGVHTFPAVLQSSGLYSLSSVVTVPSSSLGTKTYTCNVDHKPSNTKVDKRVESKYGPPCPPCPAPEFLGGPSVFLFPPKPKDTLMISRTPEVTCVVVDVSQEDPEVQFNWYVDGVEVHNAKTKPREEQFNSTYRVVSVLTVLHQDWLNGKEYKCKVSNKGLPSSIEKTISKAKGQPREPQVYTLPPSQEEMTKNQVSLTCLVKGFYPSDIAVEWESNGQPENNYKTTPPVLDSDGSFFLYSRLTVDKSRWQEGNVFSCSVLHEALHAHYTQKSLSLSLGKGSGEDCNELPPRRNTEILTGSWSDQTYPEGTQAIYKCRPGYRSLGNIIMVCRKGEWVALNPLRKCQKKSCPNPGEIRNGQIDVPGGILFGATISFSCNTGYKLFGSTSSFCDISGSSVQWSDPLPECREIYCPAPPQIDNGIIQGERDHYGYRQSVTYACNKGFTMIGEHSIYCTVNNDEGEWSGPPPECRGKS

SEQ ID NO: 76 - protein, 191 aa, artificial sequence
EDCNELPPRRNTEILTGSWSDQTYPEGTQAIYKCRPGYRSLGNIIMVCRKGEWVALNPLRKCQKKSCPNPGEIRNGQIDVPGGILFGATISFSCNTGYKLFGSTSSFCEISGSSVQWSDPLPECREIYCPAPPQIDNGIIQGERDHYGYRQSVTYACNKGFTMIGEHSIYCTVNNDEGEWSGPPPECRGKS

SEQ ID NO: 77 - protein, 643 aa, artificial sequence
QVQLVQSGAEVKKPGASVKVSCKASGYTFTNYGMNWVRQAPGQGLEWMGWINTYTGEPTYADDFKGRFTFTLDTSTSTAYLELSSLRSEDTAVYYCARTKVPHYFAYAMDYWGQGTLVTVSSASTKGPSVFPLAPCSRSTSESTAALGCLVKDYFPEPVTVSWNSGALTSGVHTFPAVLQSSGLYSLSSVVTVPSSSLGTKTYTCNVDHKPSNTKVDKRVESKYGPPCPPCPAPEFLGGPSVFLFPPKPKDTLMISRTPEVTCVVVDVSQEDPEVQFNWYVDGVEVHNAKTKPREEQFNSTYRVVSVLTVLHQDWLNGKEYKCKVSNKGLPSSIEKTISKAKGQPREPQVYTLPPSQEEMTKNQVSLTCLVKGFYPSDIAVEWESNGQPENNYKTTPPVLDSDGSFFLYSRLTVDKSRWQEGNVFSCSVLHEALHAHYTQKSLSLSLGKGSGEDCNELPPRRNTEILTGSWSDQTYPEGTQAIYKCRPGYRSLGNIIMVCRKGEWVALNPLRKCQKKSCPNPGEIRNGQIDVPGGILFGATISFSCNTGYKLFGSTSSFCEISGSSVQWSDPLPECREIYCPAPPQIDNGIIQGERDHYGYRQSVTYACNKGFTMIGEHSIYCTVNNDEGEWSGPPPECRGKS

SEQ ID NO: 78 - protein, 191 aa, artificial sequence
EDCNELPPRRNTEILTGSWSDQTYPEGTQAIYKCRPGYRSLGNIIMVCRKGEWVALNPLRKCQKKSCPNPGEIRNGQIDVPGGILFGATISFSCNTGYKLFGSTSSFCLTSGSSVQWSDPLPECREIYCPAPPQIDNGIIQGERDHYGYRQSVTYACNKGFTMIGEHSIYCTVNNDEGEWSGPPPECRGKS

SEQ ID NO: 79 - protein, 643 aa, artificial sequence
QVQLVQSGAEVKKPGASVKVSCKASGYTFTNYGMNWVRQAPGQGLEWMGWINTYTGEPTYADDFKGRFTFTLDTSTSTAYLELSSLRSEDTAVYYCARTKVPHYFAYAMDYWGQGTLVTVSSASTKGPSVFPLAPCSRSTSESTAALGCLVKDYFPEPVTVSWNSGALTSGVHTFPAVLQSSGLYSLSSVVTVPSSSLGTKTYTCNVDHKPSNTKVDKRVESKYGPPCPPCPAPEFLGGPSVFLFPPKPKDTLMISRTPEVTCVVVDVSQEDPEVQFNWYVDGVEVHNAKTKPREEQFNSTYRVVSVLTVLHQDWLNGKEYKCKVSNKGLPSSIEKTISKAKGQPREPQVYTLPPSQEEMTKNQVSLTCLVKGFYPSDIAVEWESNGQPENNYKTTPPVLDSDGSFFLYSRLTVDKSRWQEGNVFSCSVLHEALHAHYTQKSLSLSLGKGSGEDCNELPPRRNTEILTGSWSDQTYPEGTQAIYKCRPGYRSLGNIIMVCRKGEWVALNPLRKCQKKSCPNPGEIRNGQIDVPGGILFGATISFSCNTGYKLFGSTSSFCLTSGSSVQWSDPLPECREIYCPAPPQIDNGIIQGERDHYGYRQSVTYACNKGFTMIGEHSIYCTVNNDEGEWSGPPPECRGKS

SEQ ID NO: 80 - protein, 191 aa, artificial sequence
EDCNELPPRRNTEILTGSWSDQTYPEGTQAIYKCRPGYRSLGNIIMVCRKGEWVALNPDRKCQKKSCPNPGEIRNGQIDVPDGILFGATISFSCNTGYKLFGSTSSFCLTSGSSVQWSDPLPECREIYCPAPPQIDNGIIQGERDHYGYRQSVTYACNKGFTMIGEHSIYCTVNNDEGEWSGPPPECRGKS

SEQ ID NO: 81 - protein, 643 aa, artificial sequence
QVQLVQSGAEVKKPGASVKVSCKASGYTFTNYGMNWVRQAPGQGLEWMGWINTYTGEPTYADDFKGRFTFTLDTSTSTAYLELSSLRSEDTAVYYCARTKVPHYFAYAMDYWGQGTLVTVSSASTKGPSVFPLAPCSRSTSESTAALGCLVKDYFPEPVTVSWNSGALTSGVHTFPAVLQSSGLYSLSSVVTVPSSSLGTKTYTCNVDHKPSNTKVDKRVESKYGPPCPPCPAPEFLGGPSVFLFPPKPKDTLMISRTPEVTCVVVDVSQEDPEVQFNWYVDGVEVHNAKTKPREEQFNSTYRVVSVLTVLHQDWLNGKEYKCKVSNKGLPSSIEKTISKAKGQPREPQVYTLPPSQEEMTKNQVSLTCLVKGFYPSDIAVEWESNGQPENNYKTTPPVLDSDGSFFLYSRLTVDKSRWQEGNVFSCSVLHEALHAHYTQKSLSLSLGKGSGEDCNELPPRRNTEILTGSWSDQTYPEGTQAIYKCRPGYRSLGNIIMVCRKGEWVALNPDRKCQKKSCPNPGEIRNGQIDVPDGILFGATISFSCNTGYKLFGSTSSFCLTSGSSVQWSDPLPECREIYCPAPPQIDNGIIQGERDHYGYRQSVTYACNKGFTMIGEHSIYCTVNNDEGEWSGPPPECRGKS

SEQ ID NO: 82 - protein, 191 aa, artificial sequence
EDCNELPPRRNTEILTGSWSDQTYPEGTQAIYKCRPGYRSLGNIIMVCRKGEWVALNPSRKCQKKSCPNPGEIRNGQIDVPDGILFGATISFSCNTGYKLFGSTSSFCLTSGSSVQWSDPLPECREIYCPAPPQIDNGIIQGERDHYGYRQSVTYACNKGFTMIGEHSIYCTVNNDEGEWSGPPPECRGKS

SEQ ID NO: 83 - protein, 643 aa, artificial sequence
QVQLVQSGAEVKKPGASVKVSCKASGYTFTNYGMNWVRQAPGQGLEWMGWINTYTGEPTYADDFKGRFTFTLDTSTSTAYLELSSLRSEDTAVYYCARTKVPHYFAYAMDYWGQGTLVTVSSASTKGPSVFPLAPCSRSTSESTAALGCLVKDYFPEPVTVSWNSGALTSGVHTFPAVLQSSGLYSLSSVVTVPSSSLGTKTYTCNVDHKPSNTKVDKRVESKYGPPCPPCPAPEFLGGPSVFLFPPKPKDTLMISRTPEVTCVVVDVSQEDPEVQFNWYVDGVEVHNAKTKPREEQFNSTYRVVSVLTVLHQDWLNGKEYKCKVSNKGLPSSIEKTISKAKGQPREPQVYTLPPSQEEMTKNQVSLTCLVKGFYPSDIAVEWESNGQPENNYKTTPPVLDSDGSFFLYSRLTVDKSRWQEGNVFSCSVLHEALHAHYTQKSLSLSLGKGSGEDCNELPPRRNTEILTGSWSDQTYPEGTQAIYKCRPGYRSLGNIIMVCRKGEWVALNPSRKCQKKSCPNPGEIRNGQIDVPDGILFGATISFSCNTGYKLFGSTSSFCLTSGSSVQWSDPLPECREIYCPAPPQIDNGIIQGERDHYGYRQSVTYACNKGFTMIGEHSIYCTVNNDEGEWSGPPPECRGKS

SEQ ID NO: 84 - protein, 191 aa, artificial sequence
EDCNELPPRRNTEILTGSWSDQTYPEGTQAIYKCRPGYRSLGNIIMVCRKGEWVAENPDRKCQKKSCPNPGEIRNGQIDVPDGILFGATISFSCNTGYKLFGSTSSFCLTSGSSVQWSDPLPECREIYCPAPPQIDNGIIQGERDHYGYRQSVTYACNKGFTMIGEHSIYCTVNNDEGEWSGPPPECRGKS

SEQ ID NO: 85 - protein, 643 aa, artificial sequence
QVQLVQSGAEVKKPGASVKVSCKASGYTFTNYGMNWVRQAPGQGLEWMGWINTYTGEPTYADDFKGRFTFTLDTSTSTAYLELSSLRSEDTAVYYCARTKVPHYFAYAMDYWGQGTLVTVSSASTKGPSVFPLAPCSRSTSESTAALGCLVKDYFPEPVTVSWNSGALTSGVHTFPAVLQSSGLYSLSSVVTVPSSSLGTKTYTCNVDHKPSNTKVDKRVESKYGPPCPPCPAPEFLGGPSVFLFPPKPKDTLMISRTPEVTCVVVDVSQEDPEVQFNWYVDGVEVHNAKTKPREEQFNSTYRVVSVLTVLHQDWLNGKEYKCKVSNKGLPSSIEKTISKAKGQPREPQVYTLPPSQEEMTKNQVSLTCLVKGFYPSDIAVEWESNGQPENNYKTTPPVLDSDGSFFLYSRLTVDKSRWQEGNVFSCSVLHEALHAHYTQKSLSLSLGKGSGEDCNELPPRRNTEILTGSWSDQTYPEGTQAIYKCRPGYRSLGNIIMVCRKGEWVAENPDRKCQKKSCPNPGEIRNGQIDVPDGILFGATISFSCNTGYKLFGSTSSFCLTSGSSVQWSDPLPECREIYCPAPPQIDNGIIQGERDHYGYRQSVTYACNKGFTMIGEHSIYCTVNNDEGEWSGPPPECRGKS

SEQ ID NO: 86 - protein, 191 aa, artificial sequence
EDCNELPPRRNTEILTGSWSDQTYPEGTQAIYKCRPGYRSLGNIIMVCRKGEWVAENPSRKCQKKSCPNPGEIRNGQIDVPDGILFGATISFSCNTGYKLFGSTSSFCLTSGSSVQWSDPLPECREIYCPAPPQIDNGIIQGERDHYGYRQSVTYACNKGFTMIGEHSIYCTVNNDEGEWSGPPPECRGKS

SEQ ID NO: 87 - protein, 643 aa, artificial sequence
QVQLVQSGAEVKKPGASVKVSCKASGYTFTNYGMNWVRQAPGQGLEWMGWINTYTGEPTYADDFKGRFTFTLDTSTSTAYLELSSLRSEDTAVYYCARTKVPHYFAYAMDYWGQGTLVTVSSASTKGPSVFPLAPCSRSTSESTAALGCLVKDYFPEPVTVSWNSGALTSGVHTFPAVLQSSGLYSLSSVVTVPSSSLGTKTYTCNVDHKPSNTKVDKRVESKYGPPCPPCPAPEFLGGPSVFLFPPKPKDTLMISRTPEVTCVVVDVSQEDPEVQFNWYVDGVEVHNAKTKPREEQFNSTYRVVSVLTVLHQDWLNGKEYKCKVSNKGLPSSIEKTISKAKGQPREPQVYTLPPSQEEMTKNQVSLTCLVKGFYPSDIAVEWESNGQPENNYKTTPPVLDSDGSFFLYSRLTVDKSRWQEGNVFSCSVLHEALHAHYTQKSLSLSLGKGSGEDCNELPPRRNTEILTGSWSDQTYPEGTQAIYKCRPGYRSLGNIIMVCRKGEWVAENPSRKCQKKSCPNPGEIRNGQIDVPDGILFGATISFSCNTGYKLFGSTSSFCLTSGSSVQWSDPLPECREIYCPAPPQIDNGIIQGERDHYGYRQSVTYACNKGFTMIGEHSIYCTVNNDEGEWSGPPPECRGKS

SEQ ID NO: 88 - protein, 198 aa, artificial sequence
EDCNELPPRRNTEILTGSWSDQTYPEGTQAIYKCRPGYRSLGNIIMVCRKGEWVALNPSRKCQKKSCPNPGEIRNGQIDVPGGILFGATISFSCNTGYKLFGSTSSFCLISGSSVQWSDPLPECREIYCPAPPQIDNGIIQGERDHYGYRQSVTYACNKGFTMIGEHSIYCTVNNDEGEWSGPPPECRGKSGHHHHHH

SEQ ID NO: 89 - protein, 198 aa, artificial sequence
EDCNELPPRRNTEILTGSWSDQTYPEGTQAIYKCRPGYRSLGNIIMVCRKGEWVALNPLRKCQKKSCPNPGEIRNGQIDVPDGILFGATISFSCNTGYKLFGSTSSFCLISGSSVQWSDPLPECREIYCPAPPQIDNGIIQGERDHYGYRQSVTYACNKGFTMIGEHSIYCTVNNDEGEWSGPPPECRGKSGHHHHHH

SEQ ID NO: 90 - protein, 198 aa, artificial sequence
EDCNELPPRRNTEILTGSWSDQTYPEGTQAIYKCRPGYRSLGNIIMVCRKGEWVALNPLRKCQKKSCPNPGEIRNGQIDVPGGILFGATISFSCNTGYKLFGSTSSFCLTSGSSVQWSDPLPECREIYCPAPPQIDNGIIQGERDHYGYRQSVTYACNKGFTMIGEHSIYCTVNNDEGEWSGPPPECRGKSGHHHHHH

SEQ ID NO: 91 - protein, 198 aa, artificial sequence
EDCNELPPRRNTEILTGSWSDQTYPEGTQAIYKCRPGYRSLGNIIMVCRKGEWVALNPLRKCQKKSCPNPGEIRNGQIDVPGGILYGATISFSCNTGYKLFGSTSSFCLISGSSVQWSDPLPECREIYCPAPPQIDNGIIQGERDHYGYRQSVTYACNKGFTMIGEHSIYCTVNNDEGEWSGPPPECRGKSGHHHHHH

SEQ ID NO: 92 - protein, 198 aa, artificial sequence
EDCNELPPRRNTEILTGSWSDQTYPEGTQAIYKCRPGYRSLGNIIMVCRKGEWVALNPLRKCQKKSCPNPGEIRNGQIDVPGGILFGATISFSCNTGYKLFGSTSSECLISGSSVQWSDPLPECREIYCPAPPQIDNGIIQGERDHYGYRQSVTYACNKGFTMIGEHSIYCTVNNDEGEWSGPPPECRGKSGHHHHHH

SEQ ID NO: 93 - protein, 198 aa, artificial sequence
EDCNELPPRRNTEILTGSWSDQTYPEGTQAIYKCRPGYRSLGNIIMVCRKGEWVALNPLRKCQKKSCPNPGEIRNGQIDVPGGILFGATISFSCNTGYKLFGSTSSFCDISGSSVQWSDPLPECREIYCPAPPQIDNGIIQGERDHYGYRQSVTYACNKGFTMIGEHSIYCTVNNDEGEWSGPPPECRGKSGHHHHHH

SEQ ID NO: 94 - protein, 198 aa, artificial sequence
EDCNELPPRRNTEILTGSWSDQTYPEGTQAIYKCRPGYRSLGNIIMVCRKGEWVALNPLRKCQKKSCPNPGEIRNGQIDVPGGILFGATISFSCNTGYKLFGSTSSFCEISGSSVQWSDPLPECREIYCPAPPQIDNGIIQGERDHYGYRQSVTYACNKGFTMIGEHSIYCTVNNDEGEWSGPPPECRGKSGHHHHHH

SEQ ID NO: 95 - protein, 198 aa, artificial sequence
EDCNELPPRRNTEILTGSWSDQTYPEGTQAIYKCRPGYRSLGNIIMVCRKGEWVALNPDRKCQKKSCPNPGEIRNGQIDVPDGILFGATISFSCNTGYKLFGSTSSFCLTSGSSVQWSDPLPECREIYCPAPPQIDNGIIQGERDHYGYRQSVTYACNKGFTMIGEHSIYCTVNNDEGEWSGPPPECRGKSGHHHHHH

SEQ ID NO: 96 - protein, 198 aa, artificial sequence
EDCNELPPRRNTEILTGSWSDQTYPEGTQAIYKCRPGYRSLGNIIMVCRKGEWVALNPSRKCQKKSCPNPGEIRNGQIDVPDGILFGATISFSCNTGYKLFGSTSSFCLTSGSSVQWSDPLPECREIYCPAPPQIDNGIIQGERDHYGYRQSVTYACNKGFTMIGEHSIYCTVNNDEGEWSGPPPECRGKSGHHHHHH

SEQ ID NO: 97 - protein, 758 aa, artificial sequence
QVQLVQSGAEVKKPGASVKVSCKASGYTFTNYGMNWVRQAPGQGLEWMGWINTYTGEPTYADDFKGRFTFTLDTSTSTAYLELSSLRSEDTAVYYCARTKVPHYFAYAMDYWGQGTLVTVSSASTKGPSVFPLAPCSRSTSESTAALGCLVKDYFPEPVTVSWNSGALTSGVHTFPAVLQSSGLYSLSSVVTVPSSSLGTKTYTCNVDHKPSNTKVDKRVESKYGPPCPPCPAPEFLGGPSVFLFPPKPKDTLMISRTPEVTCVVVDVSQEDPEVQFNWYVDGVEVHNAKTKPREEQFNSTYRVVSVLTVLHQDWLNGKEYKCKVSNKGLPSSIEKTISKAKGQPREPQVYTLPPSQEEMTKNQVSLTCLVKGFYPSDIAVEWESNGQPENNYKTTPPVLDSDGSFFLYSRLTVDKSRWQEGNVFSCSVLHEALHAHYTQKSLSLSLGKGSGEDCNELPPRRNTEILTGSWSDQTYPEGTQAIYKCRPGYRSLGNIIMVCRKGEWVALNPLRKCQKRPCGHPGDTPFGTFTLTGGNVFEYGVKAVYTCNEGYQLLGEINYRECDTDGWTNDIPICEVVKCLPVTAPENGKIVSSAMEPDREYHFGQAVRFVCNSGYKIEGDEEMHCSDDGFWSKEKPKCVEISCKSPDVINGSPISQKIIYKENERFQYKCNMGYEYSERGDAVCTESGWRPLPSCEEKSCDNPYIPNGDYSPLRIKHRTGDEITYQCRNGFYPATRGNTAKCTSTGWIPAPRCTLKP